European Patent Application EP 4 442 826 A1, published October 9, 2024. Title: SYNTHETIC DNA CONSTRUCT ENCODING TRANSFER RNA. Applicant: UNIVERSITÄT HAMBURG. The sequence listing filed with the application follows.

SEQUENCE LISTING (130 sequences)

SEQ ID NO: 1 - DNA, 17 bp, synthetic construct
  source 1..17: mol_type = other DNA
tgacctaagtgtaaagt

SEQ ID NO: 2 - DNA, 18 bp, synthetic construct
  source 1..18: mol_type = other DNA
tgagatttccttcaggtt

SEQ ID NO: 3 - DNA, 31 bp, synthetic construct
  source 1..31: mol_type = other DNA
tatatagttctgtatgagaccactctttccc

SEQ ID NO: 4 - DNA, 17 bp, synthetic construct
  source 1..17: mol_type = other DNA
accataaacgtgaaatg

SEQ ID NO: 5 - DNA, 18 bp, synthetic construct
  source 1..18: mol_type = other DNA
tctttggatttgggaatc

SEQ ID NO: 6 - DNA, 31 bp, synthetic construct
  source 1..31: mol_type = other DNA
ttataagttctgtatgagaccactctttccc

SEQ ID NO: 7 - DNA, 50 bp, synthetic construct
  source 1..50: mol_type = other DNA
vnanantvhanannttnnnatranattcngdgvgnaanatabtnctvgnd

SEQ ID NO: 8 - DNA, 50 bp, synthetic construct
  source 1..50: mol_type = other DNA
gcnggdggcgngttcbbctgtnvnagcntncgdngncgtttnncntcggt

SEQ ID NO: 9 - DNA, 10 bp, synthetic construct
  source 1..10: mol_type = other DNA
gaaatgcctt

SEQ ID NO: 10 - DNA, 10 bp, synthetic construct
  source 1..10: mol_type = other DNA
gtgggaacta

SEQ ID NO: 11 - DNA, 10 bp, synthetic construct
  source 1..10: mol_type = other DNA
gtgttgcttg

SEQ ID NO: 12 - DNA, 66 bp, synthetic construct
  source 1..66: mol_type = other DNA
tgacctaagtgtaaagttgagatttccttcaggtttatatagttctgtatgagaccactctttccc

SEQ ID NO: 13 - DNA, 66 bp, synthetic construct
  source 1..66: mol_type = other DNA
accataaacgtgaaatgtctttggatttgggaatcttataagttctgtatgagaccactctttccc

SEQ ID NO: 14 - DNA, 66 bp, synthetic construct
  source 1..66: mol_type = other DNA
tgacctaagtgtaaagtnnnnnnnnnnnnnnnnnnnnnnnnnnnnnnnnnnnnnnnnnnnnnnnnn

SEQ ID NO: 15 - DNA, 66 bp, synthetic construct
  source 1..66: mol_type = other DNA
nnnnnnnnnnnnnnnnntgagatttccttcaggttnnnnnnnnnnnnnnnnnnnnnnnnnnnnnnn

SEQ ID NO: 16 - DNA, 66 bp, synthetic construct
  source 1..66: mol_type = other DNA
nnnnnnnnnnnnnnnnnnnnnnnnnnnnnnnnnnntatatagttctgtatgagaccactctttccc

SEQ ID NO: 17 - DNA, 66 bp, synthetic construct
  source 1..66: mol_type = other DNA
tgacctaagtgtaaagttgagatttccttcaggttnnnnnnnnnnnnnnnnnnnnnnnnnnnnnnn

SEQ ID NO: 18 - DNA, 66 bp, synthetic construct
  source 1..66: mol_type = other DNA
nnnnnnnnnnnnnnnnntgagatttccttcaggtttatatagttctgtatgagaccactctttccc

SEQ ID NO: 19 - DNA, 66 bp, synthetic construct
  source 1..66: mol_type = other DNA
tgacctaagtgtaaagtnnnnnnnnnnnnnnnnnntatatagttctgtatgagaccactctttccc

SEQ ID NO: 20 - DNA, 66 bp, synthetic construct
  source 1..66: mol_type = other DNA
accataaacgtgaaatgnnnnnnnnnnnnnnnnnnnnnnnnnnnnnnnnnnnnnnnnnnnnnnnnn

SEQ ID NO: 21 - DNA, 66 bp, synthetic construct
  source 1..66: mol_type = other DNA
nnnnnnnnnnnnnnnnntctttggatttgggaatcnnnnnnnnnnnnnnnnnnnnnnnnnnnnnnn

SEQ ID NO: 22 - DNA, 66 bp, synthetic construct
  source 1..66: mol_type = other DNA
nnnnnnnnnnnnnnnnnnnnnnnnnnnnnnnnnnnttataagttctgtatgagaccactctttccc

SEQ ID NO: 23 - DNA, 66 bp, synthetic construct
  source 1..66: mol_type = other DNA
accataaacgtgaaatgtctttggatttgggaatcnnnnnnnnnnnnnnnnnnnnnnnnnnnnnnn

SEQ ID NO: 24 - DNA, 66 bp, synthetic construct
  source 1..66: mol_type = other DNA
nnnnnnnnnnnnnnnnntctttggatttgggaatcttataagttctgtatgagaccactctttccc

SEQ ID NO: 25 - DNA, 66 bp, synthetic construct
  source 1..66: mol_type = other DNA
accataaacgtgaaatgnnnnnnnnnnnnnnnnnnttataagttctgtatgagaccactctttccc

SEQ ID NO: 26 - DNA, 66 bp, synthetic construct
  source 1..66: mol_type = other DNA
tgacctaagtgtaaagttctttggatttgggaatcnnnnnnnnnnnnnnnnnnnnnnnnnnnnnnn

SEQ ID NO: 27 - DNA, 66 bp, synthetic construct
  source 1..66: mol_type = other DNA
tgacctaagtgtaaagtnnnnnnnnnnnnnnnnnnttataagttctgtatgagaccactctttccc

SEQ ID NO: 28 - DNA, 66 bp, synthetic construct
  source 1..66: mol_type = other DNA
nnnnnnnnnnnnnnnnntgagatttccttcaggttttataagttctgtatgagaccactctttccc

SEQ ID NO: 29 - DNA, 66 bp, synthetic construct
  source 1..66: mol_type = other DNA
accataaacgtgaaatgtgagatttccttcaggttnnnnnnnnnnnnnnnnnnnnnnnnnnnnnnn

SEQ ID NO: 30 - DNA, 66 bp, synthetic construct
  source 1..66: mol_type = other DNA
nnnnnnnnnnnnnnnnntctttggatttgggaatctatatagttctgtatgagaccactctttccc

SEQ ID NO: 31 - DNA, 66 bp, synthetic construct
  source 1..66: mol_type = other DNA
accataaacgtgaaatgnnnnnnnnnnnnnnnnnntatatagttctgtatgagaccactctttccc

SEQ ID NO: 32 - DNA, 66 bp, synthetic construct
  source 1..66: mol_type = other DNA
tgacctaagtgtaaagttctttggatttgggaatcttataagttctgtatgagaccactctttccc

SEQ ID NO: 33 - DNA, 66 bp, synthetic construct
  source 1..66: mol_type = other DNA
accataaacgtgaaatgtgagatttccttcaggttttataagttctgtatgagaccactctttccc

SEQ ID NO: 34 - DNA, 66 bp, synthetic construct
  source 1..66: mol_type = other DNA
accataaacgtgaaatgtctttggatttgggaatctatatagttctgtatgagaccactctttccc

SEQ ID NO: 35 - DNA, 66 bp, synthetic construct
  source 1..66: mol_type = other DNA
tgacctaagtgtaaagttgagatttccttcaggttttataagttctgtatgagaccactctttccc

SEQ ID NO: 36 - DNA, 66 bp, synthetic construct
  source 1..66: mol_type = other DNA
tgacctaagtgtaaagttctttggatttgggaatctatatagttctgtatgagaccactctttccc

SEQ ID NO: 37 - DNA, 66 bp, synthetic construct
  source 1..66: mol_type = other DNA
accataaacgtgaaatgtgagatttccttcaggtttatatagttctgtatgagaccactctttccc

SEQ ID NO: 38 - DNA, 50 bp, synthetic construct
  source 1..50: mol_type = other DNA
ccatgatcccccactattaaggatatccggagaggatgctacctatcagg

SEQ ID NO: 39 - DNA, 50 bp, synthetic construct
  source 1..50: mol_type = other DNA
agaccagctgtatagcctcagaatgatccgtccggaaacccttactaggt

SEQ ID NO: 40 - DNA, 50 bp, synthetic construct
  source 1..50: mol_type = other DNA
gcatattgcagaacttgtgaagaggctttatgcgccacacactgcaagca

SEQ ID NO: 41 - DNA, 50 bp, synthetic construct
  source 1..50: mol_type = other DNA
gcaaaagcaaaagcattaagtagctttctggcataaacatattgcagctg

SEQ ID NO: 42 - DNA, 50 bp, synthetic construct
  source 1..50: mol_type = other DNA
ggttgcggtaagcattagagggctatcagcagcatcttatcgcagcggag

SEQ ID NO: 43 - DNA, 50 bp, synthetic construct
  source 1..50: mol_type = other DNA
ctgcagtataaccttgaagtaccatcacggagagaaacagtgccatctca

SEQ ID NO: 44 - DNA, 50 bp, synthetic construct
  source 1..50: mol_type = other DNA
aacgactacgtagtgttctataacaatcatgagaaattttagttctagat

SEQ ID NO: 45 - DNA, 50 bp, synthetic construct
  source 1..50: mol_type = other DNA
gctggtggcgagttccgctgtgccagcttccgttggcgtttgccatcggt

SEQ ID NO: 46 - DNA, 50 bp, synthetic construct; identical to SEQ ID NO: 45
  source 1..50: mol_type = other DNA

SEQ ID NO: 47 - DNA, 50 bp, synthetic construct; identical to SEQ ID NO: 45
  source 1..50: mol_type = other DNA

SEQ ID NO: 48 - DNA, 50 bp, synthetic construct
  source 1..50: mol_type = other DNA
atgcggccttgtgtggtggctcattgtggtgggccagaaaacgcgtgcaa

SEQ ID NO: 49 - DNA, 50 bp, synthetic construct
  source 1..50: mol_type = other DNA
gccagaggcgctggggccaggaggcgcaagccgggccctgaagccgcctc

SEQ ID NO: 50 - DNA, 50 bp, synthetic construct
  source 1..50: mol_type = other DNA
aaagaaattaggaaattcctgtggaagctggcgcgttgatgcacttcgtc

SEQ ID NO: 51 - DNA, 50 bp, synthetic construct
  source 1..50: mol_type = other DNA
caacaaacattttgcttttttaaaattgaaagaacaactgttttccgggt

SEQ ID NO: 52 - DNA, 17 bp, synthetic construct
  source 1..17: mol_type = other DNA
  misc_feature 8..10: note = anticodon
gcaggnnnnnnncctgt

SEQ ID NO: 53 - DNA, 18 bp, synthetic construct
  source 1..18: mol_type = other DNA
  misc_feature 8..11: note = 4nt anticodon
gcaggnnnnnnnncctgt

SEQ ID NO: 54 - DNA, 19 bp, synthetic construct
  source 1..19: mol_type = other DNA
  misc_feature 8..12: note = 5nt anticodon
gcaggnnnnnnnnncctgt

SEQ ID NO: 55 - DNA, 20 bp, synthetic construct
  source 1..20: mol_type = other DNA
  misc_feature 8..13: note = 6nt anticodon
gcaggnnnnnnnnnncctgt

SEQ ID NO: 56 - DNA, 17 bp, synthetic construct
  source 1..17: mol_type = other DNA
  misc_feature 8..10: note = anticodon
ttgggnnnnnnnctcaa

SEQ ID NO: 57 - DNA, 18 bp, synthetic construct
  source 1..18: mol_type = other DNA
  misc_feature 8..11: note = 4nt anticodon
ttgggnnnnnnnnctcaa

SEQ ID NO: 58 - DNA, 19 bp, synthetic construct
  source 1..19: mol_type = other DNA
  misc_feature 8..12: note = 5nt anticodon
ttgggnnnnnnnnnctcaa

SEQ ID NO: 59 - DNA, 20 bp, synthetic construct
  source 1..20: mol_type = other DNA
  misc_feature 8..13: note = 6nt anticodon
ttgggnnnnnnnnnnctcaa

SEQ ID NO: 60 - DNA, 17 bp, synthetic construct
  source 1..17: mol_type = other DNA
  misc_feature 8..10: note = anticodon
ttggannnnnnnttcaa

SEQ ID NO: 61 - DNA, 18 bp, synthetic construct
  source 1..18: mol_type = other DNA
  misc_feature 8..11: note = 4nt anticodon
ttggannnnnnnnttcaa

SEQ ID NO: 62 - DNA, 19 bp, synthetic construct
  source 1..19: mol_type = other DNA
  misc_feature 8..12: note = 5nt anticodon
ttggannnnnnnnnttcaa

SEQ ID NO: 63 - DNA, 20 bp, synthetic construct
  source 1..20: mol_type = other DNA
  misc_feature 8..13: note = 6nt anticodon
ttggannnnnnnnnnttcaa

SEQ ID NO: 64 - DNA, 17 bp, synthetic construct
  source 1..17: mol_type = other DNA
  misc_feature 8..10: note = anticodon
atggtnnnnnnnaccat

SEQ ID NO: 65 - DNA, 18 bp, synthetic construct
  source 1..18: mol_type = other DNA
  misc_feature 8..11: note = 4nt anticodon
atggtnnnnnnnnaccat

SEQ ID NO: 66 - DNA, 19 bp, synthetic construct
  source 1..19: mol_type = other DNA
  misc_feature 8..12: note = 5nt anticodon
atggtnnnnnnnnnaccat

SEQ ID NO: 67 - DNA, 20 bp, synthetic construct
  source 1..20: mol_type = other DNA
  misc_feature 8..13: note = 6nt anticodon
atggtnnnnnnnnnnaccat

SEQ ID NO: 68 - DNA, 17 bp, synthetic construct
  source 1..17: mol_type = other DNA
  misc_feature 8..10: note = anticodon
gcggannnnnnntccgc

SEQ ID NO: 69 - DNA, 18 bp, synthetic construct
  source 1..18: mol_type = other DNA
  misc_feature 8..11: note = 4nt anticodon
gcggannnnnnnntccgc

SEQ ID NO: 70 - DNA, 19 bp, synthetic construct
  source 1..19: mol_type = other DNA
  misc_feature 8..12: note = 5nt anticodon
gcggannnnnnnnntccgc

SEQ ID NO: 71 - DNA, 20 bp, synthetic construct
  source 1..20: mol_type = other DNA
  misc_feature 8..13: note = 6nt anticodon
gcggannnnnnnnnntccgc

SEQ ID NO: 72 - DNA, 17 bp, synthetic construct
  source 1..17: mol_type = other DNA
  misc_feature 8..10: note = anticodon
gcggtnnnnnnnaccgc

SEQ ID NO: 73 - DNA, 18 bp, synthetic construct
  source 1..18: mol_type = other DNA
  misc_feature 8..11: note = 4nt anticodon
gcggtnnnnnnnnaccgc

SEQ ID NO: 74 - DNA, 19 bp, synthetic construct
  source 1..19: mol_type = other DNA
  misc_feature 8..12: note = 5nt anticodon
gcggtnnnnnnnnnaccgc

SEQ ID NO: 75 - DNA, 20 bp, synthetic construct
  source 1..20: mol_type = other DNA
  misc_feature 8..13: note = 6nt anticodon
gcggtnnnnnnnnnnaccgc

SEQ ID NO: 76 - DNA, 17 bp, synthetic construct
  source 1..17: mol_type = other DNA
  misc_feature 8..10: note = anticodon
ggcggnnnnnnnccgcc

SEQ ID NO: 77 - DNA, 18 bp, synthetic construct
  source 1..18: mol_type = other DNA
  misc_feature 8..11: note = 4nt anticodon
ggcggnnnnnnnnccgcc

SEQ ID NO: 78 - DNA, 19 bp, synthetic construct
  source 1..19: mol_type = other DNA
  misc_feature 8..12: note = 5nt anticodon
ggcggnnnnnnnnnccgcc

SEQ ID NO: 79 - DNA, 20 bp, synthetic construct
  source 1..20: mol_type = other DNA
  misc_feature 8..13: note = 6nt anticodon
ggcggnnnnnnnnnnccgcc

SEQ ID NO: 80 - DNA, 17 bp, synthetic construct
  source 1..17: mol_type = other DNA
  misc_feature 8..10: note = anticodon
ggcgcnnnnnnngcgcc

SEQ ID NO: 81 - DNA, 18 bp, synthetic construct
  source 1..18: mol_type = other DNA
  misc_feature 8..11: note = 4nt anticodon
ggcgcnnnnnnnngcgcc

SEQ ID NO: 82 - DNA, 19 bp, synthetic construct
  source 1..19: mol_type = other DNA
  misc_feature 8..12: note = 5nt anticodon
ggcgcnnnnnnnnngcgcc

SEQ ID NO: 83 - DNA, 20 bp, synthetic construct
  source 1..20: mol_type = other DNA
  misc_feature 8..13: note = 6nt anticodon
ggcgcnnnnnnnnnngcgcc

SEQ ID NO: 84 - DNA, 17 bp, synthetic construct
  source 1..17: mol_type = other DNA
  misc_feature 8..10: note = anticodon
gcaggctnnnaacctgt

SEQ ID NO: 85 - DNA, 18 bp, synthetic construct
  source 1..18: mol_type = other DNA
  misc_feature 8..11: note = 4nt anticodon
gcaggctnnnnaacctgt

SEQ ID NO: 86 - DNA, 19 bp, synthetic construct
  source 1..19: mol_type = other DNA
  misc_feature 8..12: note = 5nt anticodon
gcaggctnnnnnaacctgt

SEQ ID NO: 87 - DNA, 20 bp, synthetic construct
  source 1..20: mol_type = other DNA
  misc_feature 8..13: note = 6nt anticodon
gcaggctnnnnnnaacctgt

SEQ ID NO: 88 - DNA, 17 bp, synthetic construct
  source 1..17: mol_type = other DNA
  misc_feature 8..10: note = anticodon
ttgggctnnnaactcaa

SEQ ID NO: 89 - DNA, 18 bp, synthetic construct
  source 1..18: mol_type = other DNA
  misc_feature 8..11: note = 4nt anticodon
ttgggctnnnnaactcaa

SEQ ID NO: 90 - DNA, 19 bp, synthetic construct
  source 1..19: mol_type = other DNA
  misc_feature 8..12: note = 5nt anticodon
ttgggctnnnnnaactcaa

SEQ ID NO: 91 - DNA, 20 bp, synthetic construct
  source 1..20: mol_type = other DNA
  misc_feature 8..13: note = 6nt anticodon
ttgggctnnnnnnaactcaa

SEQ ID NO: 92 - DNA, 17 bp, synthetic construct
  source 1..17: mol_type = other DNA
  misc_feature 8..10: note = anticodon
ttggactnnnaattcaa

SEQ ID NO: 93 - DNA, 18 bp, synthetic construct
  source 1..18: mol_type = other DNA
  misc_feature 8..11: note = 4nt anticodon
ttggactnnnnaattcaa

SEQ ID NO: 94 - DNA, 19 bp, synthetic construct
  source 1..19: mol_type = other DNA
  misc_feature 8..12: note = 5nt anticodon
ttggactnnnnnaattcaa

SEQ ID NO: 95 - DNA, 20 bp, synthetic construct
  source 1..20: mol_type = other DNA
  misc_feature 8..13: note = 6nt anticodon
ttggactnnnnnnaattcaa

SEQ ID NO: 96 - DNA, 17 bp, synthetic construct
  source 1..17: mol_type = other DNA
  misc_feature 8..10: note = anticodon
atggtctnnnaaaccat

SEQ ID NO: 97 - DNA, 18 bp, synthetic construct
  source 1..18: mol_type = other DNA
  misc_feature 8..11: note = 4nt anticodon
atggtctnnnnaaaccat

SEQ ID NO: 98 - DNA, 19 bp, synthetic construct
  source 1..19: mol_type = other DNA
  misc_feature 8..12: note = 5nt anticodon
atggtctnnnnnaaaccat

SEQ ID NO: 99 - DNA, 20 bp, synthetic construct
  source 1..20: mol_type = other DNA
  misc_feature 8..13: note = 6nt anticodon
atggtctnnnnnnaaaccat

SEQ ID NO: 100 - DNA, 17 bp, synthetic construct
  source 1..17: mol_type = other DNA
  misc_feature 8..10: note = anticodon
gcggactnnnaatccgc

SEQ ID NO: 101 - DNA, 18 bp, synthetic construct
  source 1..18: mol_type = other DNA
  misc_feature 8..11: note = 4nt anticodon
gcggactnnnnaatccgc

SEQ ID NO: 102 - DNA, 19 bp, synthetic construct
  source 1..19: mol_type = other DNA
  misc_feature 8..12: note = 5nt anticodon
gcggactnnnnnaatccgc

SEQ ID NO: 103 - DNA, 20 bp, synthetic construct
  source 1..20: mol_type = other DNA
  misc_feature 8..13: note = 6nt anticodon
gcggactnnnnnnaatccgc

SEQ ID NO: 104 - DNA, 17 bp, synthetic construct
  source 1..17: mol_type = other DNA
  misc_feature 8..10: note = anticodon
gcggtctnnnaaaccgc

SEQ ID NO: 105 - DNA, 18 bp, synthetic construct
  source 1..18: mol_type = other DNA
  misc_feature 8..11: note = 4nt anticodon
gcggtctnnnnaaaccgc

SEQ ID NO: 106 - DNA, 19 bp, synthetic construct
  source 1..19: mol_type = other DNA
  misc_feature 8..12: note = 5nt anticodon
gcggtctnnnnnaaaccgc

SEQ ID NO: 107 - DNA, 20 bp, synthetic construct
  source 1..20: mol_type = other DNA
  misc_feature 8..13: note = 6nt anticodon
gcggtctnnnnnnaaaccgc

SEQ ID NO: 108 - DNA, 17 bp, synthetic construct
  source 1..17: mol_type = other DNA
  misc_feature 8..10
ggcggctnnnaaccgcc

SEQ ID NO: 109 - DNA, 18 bp, synthetic construct
  source 1..18: mol_type = other DNA
  misc_feature 8..11: note = 4nt anticodon
ggcggctnnnnaaccgcc

SEQ ID NO: 110 - DNA, 19 bp, synthetic construct
  source 1..19: mol_type = other DNA
  misc_feature 8..12: note = 5nt anticodon
ggcggctnnnnnaaccgcc

SEQ ID NO: 111 - DNA, 20 bp, synthetic construct
  source 1..20: mol_type = other DNA
  misc_feature 8..13: note = 6nt anticodon
ggcggctnnnnnnaaccgcc

SEQ ID NO: 112 - DNA, 17 bp, synthetic construct
  source 1..17: mol_type = other DNA
  misc_feature 8..10: note = anticodon
ggcgcctnnnaagcgcc

SEQ ID NO: 113 - DNA, 18 bp, synthetic construct
  source 1..18: mol_type = other DNA
  misc_feature 8..11: note = 4nt anticodon
ggcgcctnnnnaagcgcc

SEQ ID NO: 114 - DNA, 19 bp, synthetic construct
  source 1..19: mol_type = other DNA
  misc_feature 8..12: note = 5nt anticodon
ggcgcctnnnnnaagcgcc

SEQ ID NO: 115 - DNA, 20 bp, synthetic construct
  source 1..20: mol_type = other DNA
  misc_feature 8..13: note = 6nt anticodon
ggcgcctnnnnnnaagcgcc

SEQ ID NO: 116 - DNA, 12 bp, synthetic construct
  source 1..12: mol_type = other DNA
tggggtttcccc

SEQ ID NO: 117 - DNA, 12 bp, synthetic construct
  source 1..12: mol_type = other DNA
aggggaaacccc

SEQ ID NO: 118 - DNA, 17 bp, synthetic construct
  source 1..17: mol_type = other DNA
  misc_feature 6..12: note = T loop
gcgggttcgaatcccgt

SEQ ID NO: 119 - DNA, 17 bp, synthetic construct
  source 1..17: mol_type = other DNA
  misc_feature 6..12: note = T loop
acgggttcgaatcccgt

SEQ ID NO: 120 - DNA, 17 bp, synthetic construct
  source 1..17: mol_type = other DNA
  misc_feature 6..12: note = T loop
gcgggttcgagtcccgt

SEQ ID NO: 121 - DNA, 17 bp, synthetic construct
  source 1..17: mol_type = other DNA
  misc_feature 6..12: note = T loop
acgggttcgagtcccgt

SEQ ID NO: 122 - DNA, 17 bp, synthetic construct
  source 1..17: mol_type = other DNA
  misc_feature 6..12: note = T loop
gtaggttcgagtcccat

SEQ ID NO: 123 - DNA, 17 bp, synthetic construct
  source 1..17: mol_type = other DNA
  misc_feature 6..12: note = T loop
gtcggttcgagtccgat

SEQ ID NO: 124 - DNA, 17 bp, synthetic construct
  source 1..17: mol_type = other DNA
  misc_feature 6..12: note = T loop
gccggttcgagtccggt

SEQ ID NO: 125 - DNA, 17 bp, synthetic construct
  source 1..17: mol_type = other DNA
  misc_feature 6..12: note = T loop
gcaggttcgagtcccgt

SEQ ID NO: 126 - DNA, 17 bp, synthetic construct
  source 1..17: mol_type = other DNA
  misc_feature 6..12: note = T loop
gccggttcgagtccggt

SEQ ID NO: 127 - RNA, 73 nt, synthetic construct
  source 1..73: mol_type = other RNA
  misc_feature 1..7: note = 5-prime part of acceptor stem
  misc_feature 10..13: note = 5-prime part of D stem
  misc_feature 22..25: note = 3-prime part of D stem
  misc_feature 27..31: note = 5-prime part of anticodon stem
  misc_feature 34..36: note = anticodon
  misc_feature 39..43: note = 3-prime part of anticodon stem
  misc_feature 49..53: note = 5-prime part of T stem
  misc_feature 61..65: note = 3-prime part of T stem
  misc_feature 66..72: note = 3-prime part of acceptor stem
ggctctgtggcgcaatggatagcgcattggacttcaaattcaaaggttgtgggttcgagtcccaccagagtcg

SEQ ID NO: 128 - RNA, 73 nt, synthetic construct
  source 1..73: mol_type = other RNA
  misc_feature 1..7: note = 5-prime part of acceptor stem
  misc_feature 10..13: note = 5-prime part of D stem
  misc_feature 27..31: note = 5-prime part of anticodon stem
  misc_feature 34..36: note = anticodon
  misc_feature 39..43: note = 3-prime part of anticodon stem
  misc_feature 49..53: note = 5-prime part of T stem
  misc_feature 61..65: note = 3-prime part of T stem
  misc_feature 66..72: note = 3-prime part of acceptor stem
  misc_feature 22..25: note = 3-prime part of D stem
ggctctgtggcgcaatggatagcgcattggacttcaaattcaaaggttgcgggttcgagtcccgtcagagtcg

SEQ ID NO: 129 - RNA, 91 nt, synthetic construct
  source 1..91: mol_type = other RNA
  misc_feature 1..7: note = 5-prime part of acceptor stem
  misc_feature 10..13: note = 5-prime part of D stem
  misc_feature 22..25: note = 3-prime part of D stem
  misc_feature 27..31: note = 5-prime part of anticodon stem
  misc_feature 34..36: note = anticodon
  intron 38..55
  misc_feature 57..61: note = 3-prime part of anticodon stem
  misc_feature 67..71: note = 5-prime part of T stem
  misc_feature 79..83: note = 3-prime part of T stem
  misc_feature 84..90: note = 3-prime part of acceptor stem
ggctctgtggcgcaatggatagcgcattggacttcaagctgagcctagtgtggtcattcaaaggttgcgggttcgagtcccgtcagagtcg

SEQ ID NO: 130 - RNA, 73 nt, synthetic construct
  source 1..73: mol_type = other RNA
  misc_feature 1..7: note = 5-prime part of acceptor stem
  misc_feature 10..13: note = 5-prime part of D stem
  misc_feature 22..25: note = 3-prime part of D stem
  misc_feature 34..36: note = anticodon
  misc_feature 27..31: note = 5-prime part of anticodon stem
  misc_feature 39..43: note = 3-prime part of anticodon stem
  misc_feature 49..53: note = 5-prime part of T stem
  misc_feature 61..65: note = 3-prime part of T stem
  misc_feature 66..72: note = 3-prime part of acceptor stem
ggcgctgtggcgcaatggatagcgcattggacttcaaattcaaaggttgcgggttcgagtcccgtcagcgtcg